European Patent Specification EP 3 882 364 B1, published August 23, 2023. Title: Novel Coronavirus Duplex Detection Kit. Applicant: Daan Gene Co., Ltd. Of Sun Yat-Sen University. The sequence listing filed with the application follows.

SEQUENCE LISTING (16 sequences)

SEQ ID NO: 1 - DNA, 22 bp, Artificial sequence
  Primer
tcaaagtagccactgtacagtc

SEQ ID NO: 2 - DNA, 19 bp, Artificial sequence
  Primer
ttagctaagagaatgtcat

SEQ ID NO: 3 - DNA, 27 bp, Artificial sequence
  Probe
agtgcacatcagtagtcttactctcag

SEQ ID NO: 4 - DNA, 18 bp, Artificial sequence
  Primer
tcttacaaccagaactca

SEQ ID NO: 5 - DNA, 20 bp, Artificial sequence
  Primer
aggtaagaacaagtcctgag

SEQ ID NO: 6 - DNA, 28 bp, Artificial sequence
  Probe
taattctttcacacgtggtgtttattac

SEQ ID NO: 7 - DNA, 19 bp, Artificial sequence
  Primer
agtattggagcaccgtgcg

SEQ ID NO: 8 - DNA, 20 bp, Artificial sequence
  Primer
gtggcggactcgccagttct

SEQ ID NO: 9 - DNA, 23 bp, Artificial sequence
  Probe
atcgtacctaggactctagcgcg

SEQ ID NO: 10 - DNA, 20 bp, Artificial sequence
  Primer
ctaaaatgtcagatgtaaag

SEQ ID NO: 11 - DNA, 20 bp, Artificial sequence
  Primer
tgtaactggacacattgagc

SEQ ID NO: 12 - DNA, 18 bp, Artificial sequence
  Primer
ttgtatcaaagtagccac

SEQ ID NO: 13 - DNA, 18 bp, Artificial sequence
  Primer
attgagcccacaatttag

SEQ ID NO: 14 - DNA, 117 bp, Artificial sequence
  Polyribonucleotide
agtattggagcaccgtgcggtcaacgtaagggagcagaggcggcagtcaaataacttcctcaaggaacaacacgtacctaggactctagcgcggactagaactggcgagtccgccac

SEQ ID NO: 15 - DNA, 148 bp, Artificial sequence
  Polyribonucleotide
tcaaagtagccactgtacagtctaaaatgtcagatgtaaagtgcacatcagtagtcttactctcagttttgcaacaactcagagtagaatcatcatctaaattgtgggctcaatgtgtccagttacacaatgacattctcttagctaa

SEQ ID NO: 16 - DNA, 144 bp, Artificial sequence
  Polyribonucleotide
tcttacaaccagaactcaattaccccggactcgccagtctgcatacactaattctttcacacgtggtgtttattaccctgacaaagttctaggactctattcagatcctcagttttacattcaactcaggacttgttcttacct